European Patent Specification EP 3 418 306 B1, published December 6, 2023. Title: IMPROVED ASSEMBLY OF BISPECIFIC ANTIBODIES. Applicant: GENENTECH, INC. ET AL. The sequence listing filed with the application follows.

SEQUENCE LISTING (1 sequence)

SEQ ID NO: 1 - protein, 6 aa, Artificial Sequence
  Synthetic sequence
  MISC_FEATURE (2)..(2): X is any amino acid residue
  MISC_FEATURE (4)..(4): X is any amino acid residue
RXRXRR